European Patent Application EP 4 273 243 A1, published November 8, 2023. Title: Nucleic acid constructs and vectors for podocyte specific expression. Applicant: FUNDACIÓ HOSPITAL UNIVERSITARI VALL D'HEBRON-INSTITUT DE RECERCA INSTITUCIÓ CATALANA DE RECERCA I ESTUDIS AVANÇATS UNIVERSITAT AUTÒNOMA DE BARCELONA. The sequence listing filed with the application follows.

SEQUENCE LISTING (20 sequences)

SEQ ID NO: 1 - DNA, 300 bp, Artificial
  promoter
aaaaacagaagttagaccagaccccttcctgcctatgattcttcaagaagcattgcatcatcaacatcaggcataagcattaataaagaccctaaataataacagagacgaaacacatcgcaaagagagttttcttttatcccctttaaaatgtaaatactcccaggaggaatcagccaacatcattaggggttaatgcatatgtagaataactagggcgtacttatataagggggtgggggcgcgttcgtcctcagtcgcgatcgaacactcgagccgagcagacgtgcctacggaccg

SEQ ID NO: 2 - DNA, 81 bp, Artificial
  core promoter SCP1
gtacttatataagggggtgggggcgcgttcgtcctcagtcgcgatcgaacactcgagccgagcagacgtgcctacggaccg

SEQ ID NO: 3 - DNA, 219 bp, Artificial
  podocyte-specific enhancer
aaaaacagaagttagaccagaccccttcctgcctatgattcttcaagaagcattgcatcatcaacatcaggcataagcattaataaagaccctaaataataacagagacgaaacacatcgcaaagagagttttcttttatcccctttaaaatgtaaatactcccaggaggaatcagccaacatcattaggggttaatgcatatgtagaataactagggc

SEQ ID NO: 4 - DNA, 260 bp, Artificial
  promoter
aaaaacagaagttagaccagaccccttcctgcctatgattcttcaagaagcattgcatcatcaacatcaggcataagcattaataaagaccctaaataataacagagacgaaacacatcgcaaagagagttttcttttatcccctttaaaatgtaaatactcccaggaggaatcagccaacatcattaggggttaatgcatatgggcgtttactatgggaggtctatataagcagagctcgtttagtgaaccgtcagatc

SEQ ID NO: 5 - DNA, 4513 bp, Artificial
  construct with the constitutive cytomegalovirus promoter and the CRB2 gene
gttgacattgattattgactagttattaatagtaatcaattacggggtcattagttcatagcccatatatggagttccgcgttacataacttacggtaaatggcccgcctggctgaccgcccaacgacccccgcccattgacgtcaataatgacgtatgttcccatagtaacgccaatagggactttccattgacgtcaatgggtggactatttacggtaaactgcccacttggcagtacatcaagtgtatcatatgccaagtacgccccctattgacgtcaatgacggtaaatggcccgcctggcattatgcccagtacatgaccttatgggactttcctacttggcagtacatctacgtattagtcatcgctattaccatggtgatgcggttttggcagtacatcaatgggcgtggatagcggtttgactcacggggatttccaagtctccaccccattgacgtcaatgggagtttgttttggcaccaaaatcaacgggactttccaaaatgtcgtaacaactccgccccattgacgcaaatgggcggtaggcgtgtacggtgggaggtctatataagcagagctcgtatacgccaccatggcactggcacgacccggcactcctgatcctcaggcactggcttccgtcctgctgctgctgctgtgggcacccgctctgtcactgctggccggaacagtgccctccgaacccccttctgcctgcgctagtgacccatgtgctcccggcactgagtgccaggcaaccgaaagcggcgggtacacatgtggccctatggagccacgggggtgcgctactcagccatgtcaccatggcgcactgtgcgtcccacagggaccagaccctaccggcttccggtgctattgcgtgcccgggtttcagggacctagatgcgagctggacatcgatgaatgcgccagcaggccttgtcaccatggcgctacctgtagaaatctggcagatagatacgaatgccactgtccactgggctatgccggggtgacatgcgagatggaagtcgacgagtgcgcaagcgccccctgtctgcatggaggctcctgtctggatggcgtggggtcttttcgctgcgtctgtgcaccaggatacggaggaacacgatgccagctggacctggatgaatgccagtcccagccttgtgctcatggcgggacttgtcatgacctggtgaatgggttcagatgcgattgtgccggaacaggctatgagggaactcactgcgagagagaagtgctggagtgcgcttctgcaccctgtgaacataacgccagttgtctggaggggctgggaagcttccggtgcctgtgctggccaggatacagtggcgagctgtgcgaagtggacgaggatgaatgcgcaagctccccatgtcagcacggaggcaggtgtctgcagcggagcgaccctgctctgtatggaggagtgcaggcagctttcccaggagccttcagctttaggcacgcagccgggttcctgtgccattgtccacccgggtttgagggagctgactgcggcgtggaggtcgatgaatgcgcaagccgaccatgtctgaacggaggacactgtcaggacctgcctaatggcttccagtgccattgtccagatggatacgcaggacctacctgcgaggaagacgtggatgaatgcctgagcgacccttgtctgcacggaggcacctgttccgatacagtggccggctatatctgccgatgtccagagacatggggaggacgagactgctccgtgcagctgaccggatgccagggacacacatgtcccctggctgcaacttgtatccctatttttgagtcaggcgtgcacagctacgtctgccattgtcctccagggacacatggacctttctgcgggcagaataccaccttcagcgtgatggccggatcaccaattcaggcaagcgtgccagctggaggacctctgggcctggccctgcgattccggactaccctgcctgcagggactctggcaacccgaaatgacaccaaggagtctctggaactggccctggtggccgctactctgcaggctaccctgtggagctattccacaactgtgctggtcctgagactgccagacctggctctgaacgatggccactggcatcaggtggaggtggtcctgcacctggccacactggagctgagactgtggcatgaaggctgccctgcaaggctgtgcgtggcaagcggaccagtcgccctggcttcaacagcaagcgccactccactgcccgctggcatctctagtgcacagctgggagacgccactttcgctggctgcctgcaggacgtgagggtcgatggacacctgctgctgccagaggatctgggagaaaacgtgctgctgggatgcgagcggagagaacagtgccggcctctgccatgcgtgcatggaggctcttgcgtggacctgtggacccactttagatgcgattgtgcccggccacatagagggcccacttgcgctgacgagatcccagcagccacctttggactgggaggagctccttcaagcgcaagcttcctgctgcaggaactgcccggccctaatctgaccgtgtctttcctgctgagaacaagggagagtgccgggctgctgctgcagtttgctaacgattccgctgcaggcctgaccgtcttcctgtctgaggggcgcattcgagcagaagtgcccggatcccctgcagtggtcctgcctgggcgctgggacgatggactgcgacacctggtcatgctgtcttttggcccagaccagctgcaggatctggggcagcacgtgcatgtcggagggcggctgctggcagctgactctcagccttggggaggaccattccggggatgcctgcaggacctgagactggatggctgtcacctgccattctttccactgcccctggataattcctctcagcccagcgaactggggggaagacagtcctggaacctgacagccggctgcgtgtccgaggacatgtgctctcctgatccatgttttaacggcgggacctgtctggtgacatggaatgacttccactgcacttgtccagcaaactttacaggacccacttgcgcacagcagctgtggtgcccaggacagccatgtctgccacctgcaacttgcgaggaagtgcccgatggattcgtgtgcgtggctgaggcaacctttcgcgaaggaccaccagcagccttcagcggacacaatgcaagttcagggcggctgctgggaggactgtcactggctttccggaccagagacagcgaagcatggctgctgcgagctgcagcaggagctctggagggcgtgtggctggcagtccgcaacggatccctggccgggggagtgcgaggaggacacggactgccaggagccgtgctgcccattcctggaccaagggtcgcagatggagcatggcatagggtgcgcctggcaatggagaggcctgctgcaaccacaagtcgatggctgctgtggctggacggagcagctactccagtggccctgcgaggactggctagcgacctgggatttctgcagggaccaggagccgtcagaatcctgctggctgagaatttcaccggatgcctgggaagggtggcactgggaggcctgcccctgcctctggcacgaccacgaccaggagcagcaccaggagcaagagagcactttgcaagctggccaggaacccctgcaccaattctgggatgcaggggagcacccgtgtgcgctccatccccttgtctgcatgacggggcctgtcgcgacctgttcgatgcctttgcttgcgcatgtggaccaggatgggagggaccaaggtgcgaagcccacgtggacccttgccatagcgccccatgtgcaagaggaaggtgccacactcatcccgatggccgatttgaatgccgatgtcctccaggattcggaggacctcgatgccgactgccagtcccctccaaagagtgttctctgaatgtgacctgcctggatggcagtccttgtgaaggcgggtcaccagctgcaaactgcagctgtctggagggactggctggacagcggtgccaggtgcctaccctgccatgtgaggccaacccttgcctgaatggaggaacatgccgagcagctggaggagtcagtgaatgcatctgtaacgctcggttctcagggcagttttgcgaggtggccaagggactgcctctgccactgcccttccctctgctggaggtggcagtcccagcagcatgcgcatgtctgctgctgctgctgctgggactgctgtctgggattctggctgcacggaaaaggcgccagagtgaaggcacctactctcccagtcagcaggaggtggccggggctcgcctggagatggatagtgtcctgaaagtcccacccgaagaacgcctgatttgagcgcgcaataaaagatctttattttcattagatctgtgtgttggttttttgtgtg

SEQ ID NO: 6 - DNA, 4498 bp, Artificial
  polynucleotide construct
aaaaacagaagttagaccagaccccttcctgcctatgattcttcaagaagcattgcatcatcaacatcaggcataagcattaataaagaccctaaataataacagagacgaaacacatcgcaaagagagttttcttttatcccctttaaaatgtaaatactcccaggaggaatcagccaacatcattaggggttaatgcatatgtagaataactagggcgtacttatataagggggtgggggcgcgttcgtcctcagtcgcgatcgaacactcgagccgagcagacgtgcctacggaccggtatacgccaccatggccctgggcacaacccttagggcctctctgctgctgctgggcctgctgacagagggcctggcccagctggccatccctgccagcgtgcctagaggattctgggctctgcctgagaacctgaccgtagtggaaggggctagcgtggaactccggtgcggcgtgagcacccccggctctgccgtgcagtgggccaaagacggcctgctgctgggacctgacccacggatccccggatttcctcgctaccggctggagggcgaccccgcaagaggcgagttccacctgcacatcgaggcatgcgacctgtccgatgatgccgaatatgagtgccaggtgggcagaagcgagatgggacctgagctggtgtctccccgggtgatcctgagcatcctggttcctccgaagttactactgctgacccctgaggccggaacaatggtgacctgggtggccggccaagagtatgtggtgaactgcgtgtccggcgacgcgaaacccgctccagatatcaccatcctgctgtcgggccagaccatctctgacatcagcgccaacgttaatgagggtagccaacagaagctgttcaccgtggaagccaccgccagagtgacccctagaagtagcgataatagacaactgctggtttgtgaagccagcagccccgccctggaagctccaatcaaggcctctttcaccgttaatgtgctgttcccccctggccctcccgtcatcgagtggcccggcctggacgagggccacgtgcgggcgggtcagagcctggaactgccttgcgtggctagaggcggaaaccctctggccacgctgcagtggctgaagaacggccagcctgtgagcaccgcctggggaaccgagcacacccaggccgtcgccagaagcgtgctggtgatgaccgttcggcccgaagaccacggcgcccagctgagctgtgaagcccacaatagcgtgtccgccggcacccaggagcacggaatcaccctccaggtgacctttcctccttctgccatcatcatcctcggcagcgccagccagacagaaaacaagaatgtgaccctgagctgtgtgtcgaagagctcgagaccaagagtgctgctgcggtggtggctgggctggcggcagctgctacctatggaagagacagtcatggatggcctccacggaggccacattagcatgagcaacctgacattcctggcccggagggaagacaacggcctgacacttacatgcgaagccttcagcgaggctttcaccaaggaaacattcaagaagtctctgatcctaaacgtgaaataccccgcccaaaaactgtggatcgagggccctcccgaaggccagaagctgcgggctggcaccagagtgagactggtgtgcctggctatcggcggcaaccctgagcctagcctgatgtggtacaaggatagcagaaccgtaaccgaaagccggctgcctcaggagagcagaagagtgcacctgggctccgtggaaaagagcggatctacctttagcagagaactggtgctggtgaccggcccaagcgataaccaggccaagttcacctgtaaagccggacagctgagcgcctcaacacagctggccgtgcagtttcctcctacaaatgtgaccatcctggccaatgcttctgccctaagacctggcgacgccctgaacctgacctgtgtgtcggtgagctctaacccccccgtgaacctgtcgtgggacaaggaaggcgaaagactggaaggcgtggccgctcctccccgtagagcgcctttcaagggcagcgctgctgccaggtctgtgctgctgcaggtgtctagccgggaccacgggcagagagtgacctgcagggcgcattccgccgagctgagagagacagttagcagcttctaccggctcaacgtcctgtacagacctgagttcctgggagaacaggtcctagttgtgaccgccgtggagcagggcgaggccctcctgcctgtgagcgtgagcgctaaccctgcccctgaggccttcaactggacatttagaggctaccggctgtcccctgctggaggcccccgccatagaattctgagctctggcgccctccatctgtggaacgtgaccagagccgacgacggtctgtatcagctgcactgtcagaacagcgaggggaccgcagaagctcgtctgcggctggacgtgcactacgctccgaccatccgggccctgcaagatcccacggaggtgaacgtgggcggaagcgtggacattgtgtgcaccgtggacgccaaccctatcctgccaggaatgttcaactgggagagactcggcgaagatgaagaggaccagtccctggacgacatggaaaaaatcagcagaggacctacaggccggctgagaatccaccacgccaaactcgcccaagccggagcttaccagtgcatcgtggataatggcgtggcccctcctgccagaagactgctgagactggttgtgagattcgccccacaggtggaacaccccactccactgaccaaggtggccgctgccggcgacagcaccagctccgctacactgcactgcagagcccggggagtgcctaacatcgtgttcacatggaccaagaacggcgtgcccctggacctgcaggacccccggtacaccgagcacacctaccaccagggtggcgtgcatagcagcctgctgaccatcgccaacgtgtccgccgcccaggactacgcccttttcacatgcaccgccacaaacgccctgggcagcgaccagacaaacatccagctggtgtccatctctcggcctgaccctccatctggcctgaaggtggtgtctctgacacctcactccgtaggcctggaatggaagccgggcttcgacggcggcctgcctcaacggttctgcatcagatacgaggctctgggcacacctggatttcactacgtggacgtcgtgcccccacaggccacaacattcaccctgaccggcctgcagccttccaccagatacagagtgtggctgctggcctccaacgccctgggagatagcggcctggccgataagggcacccagctccctatcactacccccggcctgcaccagcctagcggcgagcccgaggatcagctgcccacagagcccccttccggccctagcggccttcccctactccctgtgctgtttgctctgggaggactgctgctgctgtccaatgccagctgcgtgggaggcgtgctgtggcagagaagactgcggagactggccgaaggcattagcgagaagacggaggccggctcggaagaggacagagtgcgcaacgagtacgaggagagccaatggaccggcgagagagatacccagagcagcaccgtgtccaccaccgaggctgaaccttactaccgcagcctgagggacttcagccctcagctgcctccaacccaagaggaagtgagctacagccggggctttaccggcgaggatgaggatatggccttccccggccacctgtacgacgaggtggaaagaacataccctcctagtggcgcttggggccctctgtacgacgaggtgcagatgggcccttgggacctccactggcctgaggacacctaccaggatccccggggcatctatgatcaggtcgccggggatctggacacactggagcctgacagcctgcccttcgaactgcggggccacctggtggactacaaagaccatgacggtgattataaagatcatgatatcgattacaaggatgacgatgacaagtgaggcgcgccgataatcaacctctggattacaaaatttgtgaaagattgactggtattcttaactatgttgctccttttacgctatgtggatacgctgctttaatgcctttgtatcatgctattgcttcccgtatggctttcattttctcctccttgtataaatcctggttagttcttgccacggcggaactcatcgccgcctgccttgcccgctgctggacaggggctcggctgttgggcactgacaattccgtggtgcgcgctttatttgtgaaatttgtgatgctattgctttatttgtaaccattataagctgcaataaacaagttaacaacaacaattgcattcattttatgtttcaggttcagggggagatgtgggaggttttttaaagc

SEQ ID NO: 7 - DNA, 19 bp, Artificial
  sequence that includes the binding motifs of the transcription factors Lmx1b and Foxc2 in the NPHS2 gene promoter
ttaataaagaccctaaata

SEQ ID NO: 8 - DNA, 2359 bp, Artificial
  polynucleotide construct
aaaaacagaagttagaccagaccccttcctgcctatgattcttcaagaagcattgcatcatcaacatcaggcataagcattaataaagaccctaaataataacagagacgaaacacatcgcaaagagagttttcttttatcccctttaaaatgtaaatactcccaggaggaatcagccaacatcattaggggttaatgcatatgtagaataactagggcgtacttatataagggggtgggggcgcgttcgtcctcagtcgcgatcgaacactcgagccgagcagacgtgcctacggaccggtatacgccaccatggaagacgccaaaaacataaagaaaggcccggcgccattctatccgctagaggatggaaccgctggagagcaactgcataaggctatgaagagatacgccctggttcctggaacaattgcttttacagatgcacatatcgaggtgaacatcacgtacgcggaatacttcgaaatgtccgttcggttggcagaagctatgaaacgatatgggctgaatacaaatcacagaatcgtcgtatgcagtgaaaactctcttcaattctttatgccggtgttgggcgcgttatttatcggagttgcagttgcgcccgcgaacgacatttataatgaacgtgaattgctcaacagtatgaacatttcgcagcctaccgtagtgtttgtttccaaaaaggggttgcaaaaaattttgaacgtgcaaaaaaaattaccaataatccagaaaattattatcatggattctaaaacggattaccagggatttcagtcgatgtacacgttcgtcacatctcatctacctcccggttttaatgaatacgattttgtaccagagtcctttgatcgtgacaaaacaattgcactgataatgaactcctctggatctactgggttacctaagggtgtggcccttccgcatagaactgcctgcgtcagattctcgcatgccagagatcctatttttggcaatcaaatcattccggatactgcgattttaagtgttgttccattccatcacggttttggaatgtttactacactcggatatttgatatgtggatttcgagtcgtcttaatgtatagatttgaagaagagctgtttttacgatcccttcaggattacaaaattcaaagtgcgttgctagtaccaaccctattttcattcttcgccaaaagcactctgattgacaaatacgatttatctaatttacacgaaattgcttctgggggcgcacctctttcgaaagaagtcggggaagcggttgcaaaacgcttccatcttccagggatacgacaaggatatgggctcactgagactacatcagctattctgattacacccgagggggatgataaaccgggcgcggtcggtaaagttgttccattttttgaagcgaaggttgtggatctggataccgggaaaacgctgggcgttaatcagagaggcgaattatgtgtcagaggacctatgattatgtccggttatgtaaacaatccggaagcgaccaacgccttgattgacaaggatggatggctacattctggagacatagcttactgggacgaagacgaacacttcttcatagttgaccgcttgaagtctttaattaaatacaaaggataccaggtggcccccgctgaattggagtcgatattgttacaacaccccaacatcttcgacgcgggcgtggcaggtcttcccgacgatgacgccggtgaacttcccgccgccgttgttgttttggagcacggaaagacgatgacggaaaaagagatcgtggattacgtcgccagtcaagtaacaaccgcgaaaaagttgcgcggaggagttgtgtttgtggacgaagtaccgaaaggtcttaccggaaaactcgacgcaagaaaaatcagagagatcctcataaaggccaagaagggcggaaagtccaaattgtaaggcgcgccgataatcaacctctggattacaaaatttgtgaaagattgactggtattcttaactatgttgctccttttacgctatgtggatacgctgctttaatgcctttgtatcatgctattgcttcccgtatggctttcattttctcctccttgtataaatcctggttagttcttgccacggcggaactcatcgccgcctgccttgcccgctgctggacaggggctcggctgttgggcactgacaattccgtggtgcgcgctttatttgtgaaatttgtgatgctattgctttatttgtaaccattataagctgcaataaacaagttaacaacaacaattgcattcattttatgtttcaggttcagggggagatgtgggaggttttttaaagc

SEQ ID NO: 9 - DNA, 2293 bp, Artificial
  polynucleotide construct
aaaaacagaagttagaccagaccccttcctgcctatgattcttcaagaagcattgcatcatcaacatcaggcataagcattaataaagaccctaaataataacagagacgaaacacatcgcaaagagagttttcttttatcccctttaaaatgtaaatactcccaggaggaatcagccaacatcattaggggttaatgcatatgtagaataactagggcgtacttatataagggggtgggggcgcgttcgtcctcagtcgcgatcgaacactcgagccgagcagacgtgcctacggaccggtatacgccaccatggaagacgccaaaaacataaagaaaggcccggcgccattctatccgctagaggatggaaccgctggagagcaactgcataaggctatgaagagatacgccctggttcctggaacaattgcttttacagatgcacatatcgaggtgaacatcacgtacgcggaatacttcgaaatgtccgttcggttggcagaagctatgaaacgatatgggctgaatacaaatcacagaatcgtcgtatgcagtgaaaactctcttcaattctttatgccggtgttgggcgcgttatttatcggagttgcagttgcgcccgcgaacgacatttataatgaacgtgaattgctcaacagtatgaacatttcgcagcctaccgtagtgtttgtttccaaaaaggggttgcaaaaaattttgaacgtgcaaaaaaaattaccaataatccagaaaattattatcatggattctaaaacggattaccagggatttcagtcgatgtacacgttcgtcacatctcatctacctcccggttttaatgaatacgattttgtaccagagtcctttgatcgtgacaaaacaattgcactgataatgaactcctctggatctactgggttacctaagggtgtggcccttccgcatagaactgcctgcgtcagattctcgcatgccagagatcctatttttggcaatcaaatcattccggatactgcgattttaagtgttgttccattccatcacggttttggaatgtttactacactcggatatttgatatgtggatttcgagtcgtcttaatgtatagatttgaagaagagctgtttttacgatcccttcaggattacaaaattcaaagtgcgttgctagtaccaaccctattttcattcttcgccaaaagcactctgattgacaaatacgatttatctaatttacacgaaattgcttctgggggcgcacctctttcgaaagaagtcggggaagcggttgcaaaacgcttccatcttccagggatacgacaaggatatgggctcactgagactacatcagctattctgattacacccgagggggatgataaaccgggcgcggtcggtaaagttgttccattttttgaagcgaaggttgtggatctggataccgggaaaacgctgggcgttaatcagagaggcgaattatgtgtcagaggacctatgattatgtccggttatgtaaacaatccggaagcgaccaacgccttgattgacaaggatggatggctacattctggagacatagcttactgggacgaagacgaacacttcttcatagttgaccgcttgaagtctttaattaaatacaaaggataccaggtggcccccgctgaattggagtcgatattgttacaacaccccaacatcttcgacgcgggcgtggcaggtcttcccgacgatgacgccggtgaacttcccgccgccgttgttgttttggagcacggaaagacgatgacggaaaaagagatcgtggattacgtcgccagtcaagtaacaaccgcgaaaaagttgcgcggaggagttgtgtttgtggacgaagtaccgaaaggtcttaccggaaaactcgacgcaagaaaaatcagagagatcctcataaaggccaagaagggcggaaagtccaaattgtaaggcgcgccgataatcaacctctggattacaaaatttgtgaaagattgactggtattcttaactatgttgctccttttacgctatgtggatacgctgctttaatgcctttgtatcatgctattgcttcccgtatggctttcattttctcctccttgtataaatcctggttagttcttgccacggcggaactcatcgccgcctgccttgcccgctgctggacaggggctcggctgttgggcactgacaattccgtggtgcgcgctgttgcaccatgtgcttctgtaaatagtgtattgtgtttttaatgttttactggttttaataaagc

SEQ ID NO: 10 - DNA, 1390 bp, Artificial
  polynucleotide construct
aaaaacagaagttagaccagaccccttcctgcctatgattcttcaagaagcattgcatcatcaacatcaggcataagcattaataaagaccctaaataataacagagacgaaacacatcgcaaagagagttttcttttatcccctttaaaatgtaaatactcccaggaggaatcagccaacatcattaggggttaatgcatatgtagaataactagggcgtacttatataagggggtgggggcgcgttcgtcctcagtcgcgatcgaacactcgagccgagcagacgtgcctacggaccggtatacgccaccatgcccgccatgaagatcgagtgccgcatcaccggcaccctgaacggcgtggagttcgagctggtgggcggcggagagggcacccccgagcagggccgcatgaccaacaagatgaagagcaccaaaggcgccctgaccttcagcccctacctgctgagccacgtgatgggctacggcttctaccacttcggcacctaccccagcggctacgagaaccccttcctgcacgccatcaacaacggcggctacaccaacacccgcatcgagaagtacgaggacggcggcgtgctgcacgtgagcttcagctaccgctacgaggccggccgcgtgatcggcgacttcaaggtggtgggcaccggcttccccgaggacagcgtgatcttcaccgacaagatcatccgcagcaacgccaccgtggagcacctgcaccccatgggcgataacgtgctggtgggcagcttcgcccgcaccttcagcctgcgcgacggcggctactacagcttcgtggtggacagccacatgcacttcaagagcgccatccaccccagcatcctgcagaacgggggccccatgttcgccttccgccgcgtggaggagctgcacagcaacaccgagctgggcatcgtggagtaccagcacgccttcaagacccccatcgccttcgccagatctcgagctcgatgaggcgcgccgataatcaacctctggattacaaaatttgtgaaagattgactggtattcttaactatgttgctccttttacgctatgtggatacgctgctttaatgcctttgtatcatgctattgcttcccgtatggctttcattttctcctccttgtataaatcctggttagttcttgccacggcggaactcatcgccgcctgccttgcccgctgctggacaggggctcggctgttgggcactgacaattccgtggtgcgcgctttatttgtgaaatttgtgatgctattgctttatttgtaaccattataagctgcaataaacaagttaacaacaacaattgcattcattttatgtttcaggttcagggggagatgtgggaggttttttaaagc

SEQ ID NO: 11 - DNA, 1350 bp, Artificial
  polynucleotide construct
aaaaacagaagttagaccagaccccttcctgcctatgattcttcaagaagcattgcatcatcaacatcaggcataagcattaataaagaccctaaataataacagagacgaaacacatcgcaaagagagttttcttttatcccctttaaaatgtaaatactcccaggaggaatcagccaacatcattaggggttaatgcatatgggcgtttactatgggaggtctatataagcagagctcgtttagtgaaccgtcagatcgtatacgccaccatgcccgccatgaagatcgagtgccgcatcaccggcaccctgaacggcgtggagttcgagctggtgggcggcggagagggcacccccgagcagggccgcatgaccaacaagatgaagagcaccaaaggcgccctgaccttcagcccctacctgctgagccacgtgatgggctacggcttctaccacttcggcacctaccccagcggctacgagaaccccttcctgcacgccatcaacaacggcggctacaccaacacccgcatcgagaagtacgaggacggcggcgtgctgcacgtgagcttcagctaccgctacgaggccggccgcgtgatcggcgacttcaaggtggtgggcaccggcttccccgaggacagcgtgatcttcaccgacaagatcatccgcagcaacgccaccgtggagcacctgcaccccatgggcgataacgtgctggtgggcagcttcgcccgcaccttcagcctgcgcgacggcggctactacagcttcgtggtggacagccacatgcacttcaagagcgccatccaccccagcatcctgcagaacgggggccccatgttcgccttccgccgcgtggaggagctgcacagcaacaccgagctgggcatcgtggagtaccagcacgccttcaagacccccatcgccttcgccagatctcgagctcgatgaggcgcgccgataatcaacctctggattacaaaatttgtgaaagattgactggtattcttaactatgttgctccttttacgctatgtggatacgctgctttaatgcctttgtatcatgctattgcttcccgtatggctttcattttctcctccttgtataaatcctggttagttcttgccacggcggaactcatcgccgcctgccttgcccgctgctggacaggggctcggctgttgggcactgacaattccgtggtgcgcgctttatttgtgaaatttgtgatgctattgctttatttgtaaccattataagctgcaataaacaagttaacaacaacaattgcattcattttatgtttcaggttcagggggagatgtgggaggttttttaaagc

SEQ ID NO: 12 - DNA, 248 bp, Woodchuck hepatitis B virus
  Woodchuck hepatitis postranscription regulatory element  3 (WPRE3) (1)..(248)
gataatcaacctctggattacaaaatttgtgaaagattgactggtattcttaactatgttgctccttttacgctatgtggatacgctgctttaatgcctttgtatcatgctattgcttcccgtatggctttcattttctcctccttgtataaatcctggttagttcttgccacggcggaactcatcgccgcctgccttgcccgctgctggacaggggctcggctgttgggcactgacaattccgtggt

SEQ ID NO: 13 - DNA, 204 bp, Artificial
  podocyte-specific enhancer
aaaaacagaagttagaccagaccccttcctgcctatgattcttcaagaagcattgcatcatcaacatcaggcataagcattaataaagaccctaaataataacagagacgaaacacatcgcaaagagagttttcttttatcccctttaaaatgtaaatactcccaggaggaatcagccaacatcattaggggttaatgcatatg

SEQ ID NO: 14 - DNA, 1950 bp, Artificial
  polynucleotide construct
cattgcatcatcaacatcaggcataagcattaataaagaccctaaataataacagagacgaaacacatcgcaaagagagttttcttttatcccctttaaaatgtaaatactcccaggaggaatcagccaacatcattaggggttaatgcatatgtagaataactagggccaggatataaaataagaaatacgtagggaggagagaaaggcatccttgagacgactccaagaaggaaagttggggatgaggcgaaatttctgattttaccttaaagtgaccctaattcgatgaccttttgtggtttttttcttttttcttttttcttttttacttggccctgcccaagcaggacctaaaaacaaacagacaaaaaaggttactaacaactgttcctctccacgaaaatctgcagtaaaaggtaaaagatgtattcgttttgaagagaaaccagagcttgcgatgagcttctgtatctccgtcagccctctagcatgacattaggaaccctccaggagatgagtcttcacagcccgggttggcacctgcagacacgcacttttcaacgcccgcaccctgcccggggccggctctcccacccaggcctctctctgcttcagcgccgccccggccgtgggagtcggcgggcgcagtccacagctccaccaagacacagctgtcggggttccgggtgcgccccgcccgcggccccggtgtcccgcccctcgccctcagcccccacccgacggtctttagggtcccccgggcacgccacgcggacccgcagcgactccacagggactgcgctcccgtgcccctagcgctcccgcgctgctgctccagccgcccggcagctctgagggtatacgccaccatgcccgccatgaagatcgagtgccgcatcaccggcaccctgaacggcgtggagttcgagctggtgggcggcggagagggcacccccgagcagggccgcatgaccaacaagatgaagagcaccaaaggcgccctgaccttcagcccctacctgctgagccacgtgatgggctacggcttctaccacttcggcacctaccccagcggctacgagaaccccttcctgcacgccatcaacaacggcggctacaccaacacccgcatcgagaagtacgaggacggcggcgtgctgcacgtgagcttcagctaccgctacgaggccggccgcgtgatcggcgacttcaaggtggtgggcaccggcttccccgaggacagcgtgatcttcaccgacaagatcatccgcagcaacgccaccgtggagcacctgcaccccatgggcgataacgtgctggtgggcagcttcgcccgcaccttcagcctgcgcgacggcggctactacagcttcgtggtggacagccacatgcacttcaagagcgccatccaccccagcatcctgcagaacgggggccccatgttcgccttccgccgcgtggaggagctgcacagcaacaccgagctgggcatcgtggagtaccagcacgccttcaagacccccatcgccttcgccagatctcgagctcgatgaggcgcgccgataatcaacctctggattacaaaatttgtgaaagattgactggtattcttaactatgttgctccttttacgctatgtggatacgctgctttaatgcctttgtatcatgctattgcttcccgtatggctttcattttctcctccttgtataaatcctggttagttcttgccacggcggaactcatcgccgcctgccttgcccgctgctggacaggggctcggctgttgggcactgacaattccgtggtgcgcgctttatttgtgaaatttgtgatgctattgctttatttgtaaccattataagctgcaataaacaagttaacaacaacaattgcattcattttatgtttcaggttcagggggagatgtgggaggttttttaaagc

SEQ ID NO: 15 - DNA, 3686 bp, Artificial
  polynucleotide construct
gccctcctatttagtctctctgccacctacaaattgagaaagtcaaatttagtaagtccttatagtttccagctctaaaacaacaggatttgtaacatcatgtagtgccaatcaattccagcctttccattaaataatccaaatgaatcagtattcatgcattcacttattcatatggatataatacttcaaaacactaactgggaataagtgtaatactttagaaagccttgcactctttcataatctttcaccttggaaacataaaagtaaacagctttaattgatcctccctttcttctagtaacccagttcccacagatgtcagtttcttaacaaatccaaacaaggagtaaagtattgagagtttcagaatgtgtgcatatcatattttcagcaaagggatgagcaacactttcaattaaaaaggaatctaaaagaaaacagcagcatccttgtaaaagtagatgaggacagccagctggacttagctgctaactcagcactcccttccccaactcctccaccttccagccatgctgcattgacctttttatcatggaatggtatgcagcttctctgattttgtcattgtcactcataatcccagcagacttgtgttataagcagctgcttatattgctgttatgtatagatatagaaatgtaacttgtcagtggtcaaagaagccaaggaaactgagcaaaggtgactgagaacaagtgctcagcatgggctccaacacccagtagggccttttctcattgatttttctcctacaaggaatttctctcttattgaaagacagtacagtttggggaatatcatttgaccagatatcctgctccattcttggaatgaaaaacaggtgcaattttagtataagagtctagctagggatgcggatgaaattaatttataacaggaccaggctgaggaaaaacaccaataaatgctacaaatagtttgtcactttttctaacagggaaatctctaaaggatgataaagatgctagctgtgtttaatagcaaatgttaatttgggggaatatgaaataatcatgatatctttctctctttgagccaaacgcagctttggaatttttctcactgtagtgttgtaggcagaaactatcaactgaggcaggcccttgcgaggaaatatttatcctccttagcccatgcaatgatcaggtttagacagtaaaaaatctatttaagtgactggattgctcatcttttatttactttactcccagtggcctaacctggaacatatagaagaaagtagtggaatggtttttccagacgcacttcagttacttcaggtcctcagtgtttaataaggttttgggagagaaaaaaagctattgctgtgtgaattcaataaatatttaaaaaatttaaaaaatcagtgagcattatttctgccatcatgtgatctgaactatctgagtagtatcataaatcttgggtgatgggttaccttgaccaacctccctttcagtaagaaacaaattattaacagaaagtgaaagagaaataaacctattcaatgtttcaagtccctcagaagagggtgaggcagctccccagatcgttgctagatccagcctggccaatgaaccctgaaaaagcccaactcctgctttcatcatggaagcacgggacaaagtgtctcttcctaaaaacagaagttagaccagaccccttcctgcctatgattcttcaagaagcattgcatcatcaacatcaggcataagcattaataaagaccctaaataataacagagacgaaacacatcgcaaagagagttttcttttatcccctttaaaatgtaaatactcccaggaggaatcagccaacatcattaggggttaatgcatatgtagaataactagggccaggatataaaataagaaatacgtagggaggagagaaaggcatccttgagacgactccaagaaggaaagttggggatgaggcgaaatttctgattttaccttaaagtgaccctaattcgatgaccttttgtggtttttttcttttttcttttttcttttttacttggccctgcccaagcaggacctaaaaacaaacagacaaaaaaggttactaacaactgttcctctccacgaaaatctgcagtaaaaggtaaaagatgtattcgttttgaagagaaaccagagcttgcgatgagcttctgtatctccgtcagccctctagcatgacattaggaaccctccaggagatgagtcttcacagcccgggttggcacctgcagacacgcacttttcaacgcccgcaccctgcccggggccggctctcccacccaggcctctctctgcttcagcgccgccccggccgtgggagtcggcgggcgcagtccacagctccaccaagacacagctgtcggggttccgggtgcgccccgcccgcggccccggtgtcccgcccctcgccctcagcccccacccgacggtctttagggtcccccgggcacgccacgcggacccgcagcgactccacagggactgcgctcccgtgcccctagcgctcccgcgctgctgctccagccgcccggcagctctgagggtatacgccaccatgcccgccatgaagatcgagtgccgcatcaccggcaccctgaacggcgtggagttcgagctggtgggcggcggagagggcacccccgagcagggccgcatgaccaacaagatgaagagcaccaaaggcgccctgaccttcagcccctacctgctgagccacgtgatgggctacggcttctaccacttcggcacctaccccagcggctacgagaaccccttcctgcacgccatcaacaacggcggctacaccaacacccgcatcgagaagtacgaggacggcggcgtgctgcacgtgagcttcagctaccgctacgaggccggccgcgtgatcggcgacttcaaggtggtgggcaccggcttccccgaggacagcgtgatcttcaccgacaagatcatccgcagcaacgccaccgtggagcacctgcaccccatgggcgataacgtgctggtgggcagcttcgcccgcaccttcagcctgcgcgacggcggctactacagcttcgtggtggacagccacatgcacttcaagagcgccatccaccccagcatcctgcagaacgggggccccatgttcgccttccgccgcgtggaggagctgcacagcaacaccgagctgggcatcgtggagtaccagcacgccttcaagacccccatcgccttcgccagatctcgagctcgatgaggcgcgccgataatcaacctctggattacaaaatttgtgaaagattgactggtattcttaactatgttgctccttttacgctatgtggatacgctgctttaatgcctttgtatcatgctattgcttcccgtatggctttcattttctcctccttgtataaatcctggttagttcttgccacggcggaactcatcgccgcctgccttgcccgctgctggacaggggctcggctgttgggcactgacaattccgtggtgcgcgctttatttgtgaaatttgtgatgctattgctttatttgtaaccattataagctgcaataaacaagttaacaacaacaattgcattcattttatgtttcaggttcagggggagatgtgggaggttttttaaagc

SEQ ID NO: 16 - DNA, 1631 bp, Artificial
  polynucleotide construct
atagtaatcaattacggggtcattagttcatagcccatatatggagttccgcgttacataacttacggtaaatggcccgcctggctgaccgcccaacgacccccgcccattgacgtcaataatgacgtatgttcccatagtaacgccaatagggactttccattgacgtcaatgggtggagtatttacggtaaactgcccacttggcagtacatcaagtgtatcatatgccaagtacgccccctattgacgtcaatgacggtaaatggcccgcctggcattatgcccagtacatgaccttatgggactttcctacttggcagtacatctacgtattagtcatcgctattaccatggtgatgcggttttggcagtacatcaatgggcgtggatagcggtttgactcacggggatttccaagtctccaccccattgacgtcaatgggagtttgttttggcaccaaaatcaacgggactttccaaaatgtcgtaacaactccgccccattgacgcaaatgggcggtaggcgtgtacggtgggaggtctatataagcagagctggtttagtgaaccgtcagatccgctagcgctaccggtcgccaccatggtgagcaagggcgaggagctgttcaccggggtggtgcccatcctggtcgagctggacggcgacgtaaacggccacaagttcagcgtgtccggcgagggcgagggcgatgccacctacggcaagctgaccctgaagttcatctgcaccaccggcaagctgcccgtgccctggcccaccctcgtgaccaccctgacctacggcgtgcagtgcttcagccgctaccccgaccacatgaagcagcacgacttcttcaagtccgccatgcccgaaggctacgtccaggagcgcaccatcttcttcaaggacgacggcaactacaagacccgcgccgaggtgaagttcgagggcgacaccctggtgaaccgcatcgagctgaagggcatcgacttcaaggaggacggcaacatcctggggcacaagctggagtacaactacaacagccacaacgtctatatcatggccgacaagcagaagaacggcatcaaggtgaacttcaagatccgccacaacatcgaggacggcagcgtgcagctcgccgaccactaccagcagaacacccccatcggcgacggccccgtgctgctgcccgacaaccactacctgagcacccagtccgccctgagcaaagaccccaacgagaagcgcgatcacatggtcctgctggagttcgtgaccgccgccgggatcactctcggcatggacgagctgtacaagtccggactcagatctcgagctcaagcttcgaattctgcagtcgacggtaccgcgggcccgggatccaccggatctagataactgatcataatcagccataccacatttgtagaggttttacttgctttaaaaaacctcccacacctccccctgaacctgaaacataaaatgaatgcaattgttgttgttaacttgtttattgcagcttataatggttacaaataaagcaatagcatcacaaatttcacaaataaagcatttttttcactgcattctagttgtggtttgtccaaactcatcaatgtatctta

SEQ ID NO: 17 - DNA, 2581 bp, Artificial
  polynucleotide construct
gttgacattgattattgactagttattaatagtaatcaattacggggtcattagttcatagcccatatatggagttccgcgttacataacttacggtaaatggcccgcctggctgaccgcccaacgacccccgcccattgacgtcaataatgacgtatgttcccatagtaacgccaatagggactttccattgacgtcaatgggtggactatttacggtaaactgcccacttggcagtacatcaagtgtatcatatgccaagtacgccccctattgacgtcaatgacggtaaatggcccgcctggcattatgcccagtacatgaccttatgggactttcctacttggcagtacatctacgtattagtcatcgctattaccatggtgatgcggttttggcagtacatcaatgggcgtggatagcggtttgactcacggggatttccaagtctccaccccattgacgtcaatgggagtttgttttggcaccaaaatcaacgggactttccaaaatgtcgtaacaactccgccccattgacgcaaatgggcggtaggcgtgtacggtgggaggtctatataagcagagctcgtatacgccaccatggaagacgccaaaaacataaagaaaggcccggcgccattctatccgctagaggatggaaccgctggagagcaactgcataaggctatgaagagatacgccctggttcctggaacaattgcttttacagatgcacatatcgaggtgaacatcacgtacgcggaatacttcgaaatgtccgttcggttggcagaagctatgaaacgatatgggctgaatacaaatcacagaatcgtcgtatgcagtgaaaactctcttcaattctttatgccggtgttgggcgcgttatttatcggagttgcagttgcgcccgcgaacgacatttataatgaacgtgaattgctcaacagtatgaacatttcgcagcctaccgtagtgtttgtttccaaaaaggggttgcaaaaaattttgaacgtgcaaaaaaaattaccaataatccagaaaattattatcatggattctaaaacggattaccagggatttcagtcgatgtacacgttcgtcacatctcatctacctcccggttttaatgaatacgattttgtaccagagtcctttgatcgtgacaaaacaattgcactgataatgaactcctctggatctactgggttacctaagggtgtggcccttccgcatagaactgcctgcgtcagattctcgcatgccagagatcctatttttggcaatcaaatcattccggatactgcgattttaagtgttgttccattccatcacggttttggaatgtttactacactcggatatttgatatgtggatttcgagtcgtcttaatgtatagatttgaagaagagctgtttttacgatcccttcaggattacaaaattcaaagtgcgttgctagtaccaaccctattttcattcttcgccaaaagcactctgattgacaaatacgatttatctaatttacacgaaattgcttctgggggcgcacctctttcgaaagaagtcggggaagcggttgcaaaacgcttccatcttccagggatacgacaaggatatgggctcactgagactacatcagctattctgattacacccgagggggatgataaaccgggcgcggtcggtaaagttgttccattttttgaagcgaaggttgtggatctggataccgggaaaacgctgggcgttaatcagagaggcgaattatgtgtcagaggacctatgattatgtccggttatgtaaacaatccggaagcgaccaacgccttgattgacaaggatggatggctacattctggagacatagcttactgggacgaagacgaacacttcttcatagttgaccgcttgaagtctttaattaaatacaaaggataccaggtggcccccgctgaattggagtcgatattgttacaacaccccaacatcttcgacgcgggcgtggcaggtcttcccgacgatgacgccggtgaacttcccgccgccgttgttgttttggagcacggaaagacgatgacggaaaaagagatcgtggattacgtcgccagtcaagtaacaaccgcgaaaaagttgcgcggaggagttgtgtttgtggacgaagtaccgaaaggtcttaccggaaaactcgacgcaagaaaaatcagagagatcctcataaaggccaagaagggcggaaagtccaaattgtaaggcgcgccgataatcaacctctggattacaaaatttgtgaaagattgactggtattcttaactatgttgctccttttacgctatgtggatacgctgctttaatgcctttgtatcatgctattgcttcccgtatggctttcattttctcctccttgtataaatcctggttagttcttgccacggcggaactcatcgccgcctgccttgcccgctgctggacaggggctcggctgttgggcactgacaattccgtggtgcgcgctgttgcaccatgtgcttctgtaaatagtgtattgtgtttttaatgttttactggttttaataaagc

SEQ ID NO: 18 - DNA, 4396 bp, Artificial
  polynucleotide construct
aaaaacagaagttagaccagaccccttcctgcctatgattcttcaagaagcattgcatcatcaacatcaggcataagcattaataaagaccctaaataataacagagacgaaacacatcgcaaagagagttttcttttatcccctttaaaatgtaaatactcccaggaggaatcagccaacatcattaggggttaatgcatatgtagaataactagggcgtacttatataagggggtgggggcgcgttcgtcctcagtcgcgatcgaacactcgagccgagcagacgtgcctacggaccgtatacgccaccatggcactggcacgacccggcactcctgatcctcaggcactggcttccgtcctgctgctgctgctgtgggcacccgctctgtcactgctggccggaacagtgccctccgaacccccttctgcctgcgctagtgacccatgtgctcccggcactgagtgccaggcaaccgaaagcggcgggtacacatgtggccctatggagccacgggggtgcgctactcagccatgtcaccatggcgcactgtgcgtcccacagggaccagaccctaccggcttccggtgctattgcgtgcccgggtttcagggacctagatgcgagctggacatcgatgaatgcgccagcaggccttgtcaccatggcgctacctgtagaaatctggcagatagatacgaatgccactgtccactgggctatgccggggtgacatgcgagatggaagtcgacgagtgcgcaagcgccccctgtctgcatggaggctcctgtctggatggcgtggggtcttttcgctgcgtctgtgcaccaggatacggaggaacacgatgccagctggacctggatgaatgccagtcccagccttgtgctcatggcgggacttgtcatgacctggtgaatgggttcagatgcgattgtgccggaacaggctatgagggaactcactgcgagagagaagtgctggagtgcgcttctgcaccctgtgaacataacgccagttgtctggaggggctgggaagcttccggtgcctgtgctggccaggatacagtggcgagctgtgcgaagtggacgaggatgaatgcgcaagctccccatgtcagcacggaggcaggtgtctgcagcggagcgaccctgctctgtatggaggagtgcaggcagctttcccaggagccttcagctttaggcacgcagccgggttcctgtgccattgtccacccgggtttgagggagctgactgcggcgtggaggtcgatgaatgcgcaagccgaccatgtctgaacggaggacactgtcaggacctgcctaatggcttccagtgccattgtccagatggatacgcaggacctacctgcgaggaagacgtggatgaatgcctgagcgacccttgtctgcacggaggcacctgttccgatacagtggccggctatatctgccgatgtccagagacatggggaggacgagactgctccgtgcagctgaccggatgccagggacacacatgtcccctggctgcaacttgtatccctatttttgagtcaggcgtgcacagctacgtctgccattgtcctccagggacacatggacctttctgcgggcagaataccaccttcagcgtgatggccggatcaccaattcaggcaagcgtgccagctggaggacctctgggcctggccctgcgattccggactaccctgcctgcagggactctggcaacccgaaatgacaccaaggagtctctggaactggccctggtggccgctactctgcaggctaccctgtggagctattccacaactgtgctggtcctgagactgccagacctggctctgaacgatggccactggcatcaggtggaggtggtcctgcacctggccacactggagctgagactgtggcatgaaggctgccctgcaaggctgtgcgtggcaagcggaccagtcgccctggcttcaacagcaagcgccactccactgcccgctggcatctctagtgcacagctgggagacgccactttcgctggctgcctgcaggacgtgagggtcgatggacacctgctgctgccagaggatctgggagaaaacgtgctgctgggatgcgagcggagagaacagtgccggcctctgccatgcgtgcatggaggctcttgcgtggacctgtggacccactttagatgcgattgtgcccggccacatagagggcccacttgcgctgacgagatcccagcagccacctttggactgggaggagctccttcaagcgcaagcttcctgctgcaggaactgcccggccctaatctgaccgtgtctttcctgctgagaacaagggagagtgccgggctgctgctgcagtttgctaacgattccgctgcaggcctgaccgtcttcctgtctgaggggcgcattcgagcagaagtgcccggatcccctgcagtggtcctgcctgggcgctgggacgatggactgcgacacctggtcatgctgtcttttggcccagaccagctgcaggatctggggcagcacgtgcatgtcggagggcggctgctggcagctgactctcagccttggggaggaccattccggggatgcctgcaggacctgagactggatggctgtcacctgccattctttccactgcccctggataattcctctcagcccagcgaactggggggaagacagtcctggaacctgacagccggctgcgtgtccgaggacatgtgctctcctgatccatgttttaacggcgggacctgtctggtgacatggaatgacttccactgcacttgtccagcaaactttacaggacccacttgcgcacagcagctgtggtgcccaggacagccatgtctgccacctgcaacttgcgaggaagtgcccgatggattcgtgtgcgtggctgaggcaacctttcgcgaaggaccaccagcagccttcagcggacacaatgcaagttcagggcggctgctgggaggactgtcactggctttccggaccagagacagcgaagcatggctgctgcgagctgcagcaggagctctggagggcgtgtggctggcagtccgcaacggatccctggccgggggagtgcgaggaggacacggactgccaggagccgtgctgcccattcctggaccaagggtcgcagatggagcatggcatagggtgcgcctggcaatggagaggcctgctgcaaccacaagtcgatggctgctgtggctggacggagcagctactccagtggccctgcgaggactggctagcgacctgggatttctgcagggaccaggagccgtcagaatcctgctggctgagaatttcaccggatgcctgggaagggtggcactgggaggcctgcccctgcctctggcacgaccacgaccaggagcagcaccaggagcaagagagcactttgcaagctggccaggaacccctgcaccaattctgggatgcaggggagcacccgtgtgcgctccatccccttgtctgcatgacggggcctgtcgcgacctgttcgatgcctttgcttgcgcatgtggaccaggatgggagggaccaaggtgcgaagcccacgtggacccttgccatagcgccccatgtgcaagaggaaggtgccacactcatcccgatggccgatttgaatgccgatgtcctccaggattcggaggacctcgatgccgactgccagtcccctccaaagagtgttctctgaatgtgacctgcctggatggcagtccttgtgaaggcgggtcaccagctgcaaactgcagctgtctggagggactggctggacagcggtgccaggtgcctaccctgccatgtgaggccaacccttgcctgaatggaggaacatgccgagcagctggaggagtcagtgaatgcatctgtaacgctcggttctcagggcagttttgcgaggtggccaagggactgcctctgccactgcccttccctctgctggaggtggcagtcccagcagcatgcgcatgtctgctgctgctgctgctgggactgctgtctgggattctggctgcacggaaaaggcgccagagtgaaggcacctactctcccagtcagcaggaggtggccggggctcgcctggagatggatagtgtcctgaaagtcccacccgaagaacgcctgatttgagcgcgcagacatgataagatacattgatgagtttggacaaaccacaacaagaatgcagtgaaaaaaatgctttatttgtgaaatttgtgatgctattgctttatttgtaaccattataagctgcaataaacaagttaacaacaacaattgcattcattttatgtttcaggttcagggggagatgtgggaggttttttaaagcaagtaaaacctctacaaatgtggta

SEQ ID NO: 19 - DNA, 4241 bp, Artificial
  polynucleotide construct
aaaaacagaagttagaccagaccccttcctgcctatgattcttcaagaagcattgcatcatcaacatcaggcataagcattaataaagaccctaaataataacagagacgaaacacatcgcaaagagagttttcttttatcccctttaaaatgtaaatactcccaggaggaatcagccaacatcattaggggttaatgcatatgtagaataactagggcgtacttatataagggggtgggggcgcgttcgtcctcagtcgcgatcgaacactcgagccgagcagacgtgcctacggaccgtatacgccaccatggcactggcacgacccggcactcctgatcctcaggcactggcttccgtcctgctgctgctgctgtgggcacccgctctgtcactgctggccggaacagtgccctccgaacccccttctgcctgcgctagtgacccatgtgctcccggcactgagtgccaggcaaccgaaagcggcgggtacacatgtggccctatggagccacgggggtgcgctactcagccatgtcaccatggcgcactgtgcgtcccacagggaccagaccctaccggcttccggtgctattgcgtgcccgggtttcagggacctagatgcgagctggacatcgatgaatgcgccagcaggccttgtcaccatggcgctacctgtagaaatctggcagatagatacgaatgccactgtccactgggctatgccggggtgacatgcgagatggaagtcgacgagtgcgcaagcgccccctgtctgcatggaggctcctgtctggatggcgtggggtcttttcgctgcgtctgtgcaccaggatacggaggaacacgatgccagctggacctggatgaatgccagtcccagccttgtgctcatggcgggacttgtcatgacctggtgaatgggttcagatgcgattgtgccggaacaggctatgagggaactcactgcgagagagaagtgctggagtgcgcttctgcaccctgtgaacataacgccagttgtctggaggggctgggaagcttccggtgcctgtgctggccaggatacagtggcgagctgtgcgaagtggacgaggatgaatgcgcaagctccccatgtcagcacggaggcaggtgtctgcagcggagcgaccctgctctgtatggaggagtgcaggcagctttcccaggagccttcagctttaggcacgcagccgggttcctgtgccattgtccacccgggtttgagggagctgactgcggcgtggaggtcgatgaatgcgcaagccgaccatgtctgaacggaggacactgtcaggacctgcctaatggcttccagtgccattgtccagatggatacgcaggacctacctgcgaggaagacgtggatgaatgcctgagcgacccttgtctgcacggaggcacctgttccgatacagtggccggctatatctgccgatgtccagagacatggggaggacgagactgctccgtgcagctgaccggatgccagggacacacatgtcccctggctgcaacttgtatccctatttttgagtcaggcgtgcacagctacgtctgccattgtcctccagggacacatggacctttctgcgggcagaataccaccttcagcgtgatggccggatcaccaattcaggcaagcgtgccagctggaggacctctgggcctggccctgcgattccggactaccctgcctgcagggactctggcaacccgaaatgacaccaaggagtctctggaactggccctggtggccgctactctgcaggctaccctgtggagctattccacaactgtgctggtcctgagactgccagacctggctctgaacgatggccactggcatcaggtggaggtggtcctgcacctggccacactggagctgagactgtggcatgaaggctgccctgcaaggctgtgcgtggcaagcggaccagtcgccctggcttcaacagcaagcgccactccactgcccgctggcatctctagtgcacagctgggagacgccactttcgctggctgcctgcaggacgtgagggtcgatggacacctgctgctgccagaggatctgggagaaaacgtgctgctgggatgcgagcggagagaacagtgccggcctctgccatgcgtgcatggaggctcttgcgtggacctgtggacccactttagatgcgattgtgcccggccacatagagggcccacttgcgctgacgagatcccagcagccacctttggactgggaggagctccttcaagcgcaagcttcctgctgcaggaactgcccggccctaatctgaccgtgtctttcctgctgagaacaagggagagtgccgggctgctgctgcagtttgctaacgattccgctgcaggcctgaccgtcttcctgtctgaggggcgcattcgagcagaagtgcccggatcccctgcagtggtcctgcctgggcgctgggacgatggactgcgacacctggtcatgctgtcttttggcccagaccagctgcaggatctggggcagcacgtgcatgtcggagggcggctgctggcagctgactctcagccttggggaggaccattccggggatgcctgcaggacctgagactggatggctgtcacctgccattctttccactgcccctggataattcctctcagcccagcgaactggggggaagacagtcctggaacctgacagccggctgcgtgtccgaggacatgtgctctcctgatccatgttttaacggcgggacctgtctggtgacatggaatgacttccactgcacttgtccagcaaactttacaggacccacttgcgcacagcagctgtggtgcccaggacagccatgtctgccacctgcaacttgcgaggaagtgcccgatggattcgtgtgcgtggctgaggcaacctttcgcgaaggaccaccagcagccttcagcggacacaatgcaagttcagggcggctgctgggaggactgtcactggctttccggaccagagacagcgaagcatggctgctgcgagctgcagcaggagctctggagggcgtgtggctggcagtccgcaacggatccctggccgggggagtgcgaggaggacacggactgccaggagccgtgctgcccattcctggaccaagggtcgcagatggagcatggcatagggtgcgcctggcaatggagaggcctgctgcaaccacaagtcgatggctgctgtggctggacggagcagctactccagtggccctgcgaggactggctagcgacctgggatttctgcagggaccaggagccgtcagaatcctgctggctgagaatttcaccggatgcctgggaagggtggcactgggaggcctgcccctgcctctggcacgaccacgaccaggagcagcaccaggagcaagagagcactttgcaagctggccaggaacccctgcaccaattctgggatgcaggggagcacccgtgtgcgctccatccccttgtctgcatgacggggcctgtcgcgacctgttcgatgcctttgcttgcgcatgtggaccaggatgggagggaccaaggtgcgaagcccacgtggacccttgccatagcgccccatgtgcaagaggaaggtgccacactcatcccgatggccgatttgaatgccgatgtcctccaggattcggaggacctcgatgccgactgccagtcccctccaaagagtgttctctgaatgtgacctgcctggatggcagtccttgtgaaggcgggtcaccagctgcaaactgcagctgtctggagggactggctggacagcggtgccaggtgcctaccctgccatgtgaggccaacccttgcctgaatggaggaacatgccgagcagctggaggagtcagtgaatgcatctgtaacgctcggttctcagggcagttttgcgaggtggccaagggactgcctctgccactgcccttccctctgctggaggtggcagtcccagcagcatgcgcatgtctgctgctgctgctgctgggactgctgtctgggattctggctgcacggaaaaggcgccagagtgaaggcacctactctcccagtcagcaggaggtggccggggctcgcctggagatggatagtgtcctgaaagtcccacccgaagaacgcctgatttgagcgcgctgttgcaccatgtgcttctgtaaatagtgtattgtgtttttaatgttttactggttttaataaagc

SEQ ID NO: 20 - DNA, 56 bp, Artificial
  minimal core promoter
ggcgtttactatgggaggtctatataagcagagctcgtttagtgaaccgtcagatc